European Patent Application EP 4 527 415 A1, published March 26, 2025. Title: ANTIBODY - DRUG CONJUGATE CONTAINING PROTEIN DEGRADATION AGENT BIOACTIVE COMPOUND, METHOD FOR PREPARING SAME, AND USE THEREOF. Applicant: MEDILINK THERAPEUTICS (SUZHOU) CO., LTD. Application EP, filed May 16, 2023. The sequence listing filed with the application follows.

SEQUENCE LISTING (10 sequences)

SEQ ID NO: 1 - protein, 123 aa, synthetic construct
EGQLVESGGGLVQPGGSLRLSCAASGFTISSYWMNWVRQAPGKGLEWVANIKQDGSEKYYVDSVQGRFTISRDNAKNSLYLQMNSLRAEDTAVYYCARRMYSSGWYWGAFDMWGQGTMVTVSS

SEQ ID NO: 2 - protein, 108 aa, synthetic construct
EIVLTQSPGTLSLSPGERATLSCRASQSVSSIYLAWNQQKPGQAPRLLIYGTFKRATGIPDRFSGSGSGTDFTLTISSLEPEDFAVYYCQQYDTSSITFGQGTRLEIK

SEQ ID NO: 3 - protein, 453 aa, synthetic construct
EGQLVESGGGLVQPGGSLRLSCAASGFTISSYWMNWVRQAPGKGLEWVANIKQDGSEKYYVDSVQGRFTISRDNAKNSLYLQMNSLRAEDTAVYYCARRMYSSGWYWGAFDMWGQGTMVTVSSASTKGPSVFPLAPSSKSTSGGTAALGCLVKDYFPEPVTVSWNSGALTSGVHTFPAVLQSSGLYSLSSVVTVPSSSLGTQTYICNVNHKPSNTKVDKKVEPKSCDKTHTCPPCPAPELLGGPSVFLFPPKPKDTLMISRTPEVTCVVVDVSHEDPEVKFNWYVDGVEVHNAKTKPREEQYNSTYRVVSVLTVLHQDWLNGKEYKCKVSNKALPAPIEKTISKAKGQPREPQVYTLPPSRDELTKNQVSLTCLVKGFYPSDIAVEWESNGQPENNYKTTPPVLDSDGSFFLYSKLTVDKSRWQQGNVFSCSVMHEALHNHYTQKSLSLSPGK

SEQ ID NO: 4 - protein, 215 aa, synthetic construct
EIVLTQSPGTLSLSPGERATLSCRASQSVSSIYLAWNQQKPGQAPRLLIYGTFKRATGIPDRFSGSGSGTDFTLTISSLEPEDFAVYYCQQYDTSSITFGQGTRLEIKRTVAAPSVFIFPPSDEQLKSGTASVVCLLNNFYPREAKVQWKVDNALQSGNSQESVTEQDSKDSTYSLSSTLTLSKADYEKHKVYACEVTHQGLSSPVTKSFNRGEC

SEQ ID NO: 5 - protein, 120 aa, synthetic construct
EVQLLESGGGLVQPGGSLRLSCAASGFTFSSYAMNWVRQAPGKGLEWVSGISGSGGSTYYADSVQGRFTISRDNSKNTLYLQMNSLRAEDTAVYYCAKARSGYDYFFDYWGQGTLVTVSS

SEQ ID NO: 6 - protein, 108 aa, synthetic construct
EIVLTQSPGTLSLSPGERATLSCRASQRISSSFLAWYQQKPGQAPSLLIYGASSRATGIPDRFSGSGSGTDFTLTISSLEPEDFAVFYCQQYSNSPLTFGGGTKVEIK

SEQ ID NO: 7 - protein, 450 aa, synthetic construct
EVQLLESGGGLVQPGGSLRLSCAASGFTFSSYAMNWVRQAPGKGLEWVSGISGSGGSTYYADSVQGRFTISRDNSKNTLYLQMNSLRAEDTAVYYCAKARSGYDYFFDYWGQGTLVTVSSASTKGPSVFPLAPSSKSTSGGTAALGCLVKDYFPEPVTVSWNSGALTSGVHTFPAVLQSSGLYSLSSVVTVPSSSLGTQTYICNVNHKPSNTKVDKKVEPKSCDKTHTCPPCPAPELLGGPSVFLFPPKPKDTLMISRTPEVTCVVVDVSHEDPEVKFNWYVDGVEVHNAKTKPREEQYNSTYRVVSVLTVLHQDWLNGKEYKCKVSNKALPAPIEKTISKAKGQPREPQVYTLPPSRDELTKNQVSLTCLVKGFYPSDIAVEWESNGQPENNYKTTPPVLDSDGSFFLYSKLTVDKSRWQQGNVFSCSVMHEALHNHYTQKSLSLSPGK

SEQ ID NO: 8 - protein, 215 aa, synthetic construct
EIVLTQSPGTLSLSPGERATLSCRASQRISSSFLAWYQQKPGQAPSLLIYGASSRATGIPDRFSGSGSGTDFTLTISSLEPEDFAVFYCQQYSNSPLTFGGGTKVEIKRTVAAPSVFIFPPSDEQLKSGTASVVCLLNNFYPREAKVQWKVDNALQSGNSQESVTEQDSKDSTYSLSSTLTLSKADYEKHKVYACEVTHQGLSSPVTKSFNRGEC

SEQ ID NO: 9 - protein, 330 aa, synthetic construct [sequence omitted]

SEQ ID NO: 10 - protein, 107 aa, synthetic construct [sequence omitted]